European Patent Application EP 4 722 365 A1, published April 8, 2026. Title: 一种用于代谢疾病的双链核苷酸化合物及其应用. Applicant: 维亚臻生物技术 （苏州）有限公司. Application CN. The sequence listing filed with the application follows.

SEQUENCE LISTING (201 sequences)

SEQ ID NO: 1 - RNA, 20 nt, synthetic construct
  source 1..20: mol_type = other RNA
cgatgggtccagaagaagtt

SEQ ID NO: 2 - RNA, 20 nt, synthetic construct
  source 1..20: mol_type = other RNA
ggttatttaaaagaaattat

SEQ ID NO: 3 - RNA, 20 nt, synthetic construct
  source 1..20: mol_type = other RNA
tgctgaccaccaggaactat

SEQ ID NO: 4 - RNA, 20 nt, synthetic construct
  source 1..20: mol_type = other RNA
gaccaccaggaactatatct

SEQ ID NO: 5 - RNA, 20 nt, synthetic construct
  source 1..20: mol_type = other RNA
atgggtgtctgtgggttatt

SEQ ID NO: 6 - RNA, 20 nt, synthetic construct
  source 1..20: mol_type = other RNA
tgggtgtctgtgggttattt

SEQ ID NO: 7 - RNA, 20 nt, synthetic construct
  source 1..20: mol_type = other RNA
gggtgtctgtgggttattta

SEQ ID NO: 8 - RNA, 20 nt, synthetic construct
  source 1..20: mol_type = other RNA
gtgtctgtgggttatttaaa

SEQ ID NO: 9 - RNA, 20 nt, synthetic construct
  source 1..20: mol_type = other RNA
tgggttatttaaaagaaatt

SEQ ID NO: 10 - RNA, 20 nt, synthetic construct
  source 1..20: mol_type = other RNA
gggttatttaaaagaaatta

SEQ ID NO: 11 - RNA, 20 nt, synthetic construct
  source 1..20: mol_type = other RNA
ctgaccaccaggaactatat

SEQ ID NO: 12 - RNA, 20 nt, synthetic construct
  source 1..20: mol_type = other RNA
accaccaggaactatatctt

SEQ ID NO: 13 - RNA, 20 nt, synthetic construct
  source 1..20: mol_type = other RNA
ccaccaggaactatatcttt

SEQ ID NO: 14 - RNA, 20 nt, synthetic construct
  source 1..20: mol_type = other RNA
caggaactatatctttggat

SEQ ID NO: 15 - RNA, 20 nt, synthetic construct
  source 1..20: mol_type = other RNA
gggagtggcaatgctatcat

SEQ ID NO: 16 - RNA, 20 nt, synthetic construct
  source 1..20: mol_type = other RNA
catgggtgtctgtgggttat

SEQ ID NO: 17 - RNA, 20 nt, synthetic construct
  source 1..20: mol_type = other RNA
ggtgtctgtgggttatttaa

SEQ ID NO: 18 - RNA, 20 nt, synthetic construct
  source 1..20: mol_type = other RNA
tgtctgtgggttatttaaaa

SEQ ID NO: 19 - RNA, 20 nt, synthetic construct
  source 1..20: mol_type = other RNA
gtctgtgggttatttaaaag

SEQ ID NO: 20 - RNA, 20 nt, synthetic construct
  source 1..20: mol_type = other RNA
ctgtgggttatttaaaagaa

SEQ ID NO: 21 - RNA, 20 nt, synthetic construct
  source 1..20: mol_type = other RNA
gactactttcccatccagct

SEQ ID NO: 22 - RNA, 20 nt, synthetic construct
  source 1..20: mol_type = other RNA
ctggtgaagacacacaacct

SEQ ID NO: 23 - RNA, 20 nt, synthetic construct
  source 1..20: mol_type = other RNA
gtgaagacacacaacctgct

SEQ ID NO: 24 - RNA, 20 nt, synthetic construct
  source 1..20: mol_type = other RNA
cctgctgaccaccaggaact

SEQ ID NO: 25 - RNA, 20 nt, synthetic construct
  source 1..20: mol_type = other RNA
gctgaccaccaggaactata

SEQ ID NO: 26 - RNA, 20 nt, synthetic construct
  source 1..20: mol_type = other RNA
gaatgggagtggcaatgcta

SEQ ID NO: 27 - RNA, 20 nt, synthetic construct
  source 1..20: mol_type = other RNA
gagtggcaatgctatcatca

SEQ ID NO: 28 - RNA, 20 nt, synthetic construct
  source 1..20: mol_type = other RNA
agtggcaatgctatcatcat

SEQ ID NO: 29 - RNA, 20 nt, synthetic construct
  source 1..20: mol_type = other RNA
ggcaatgctatcatcatcgt

SEQ ID NO: 30 - RNA, 20 nt, synthetic construct
  source 1..20: mol_type = other RNA
agctccatgcctggcaagaa

SEQ ID NO: 31 - RNA, 20 nt, synthetic construct
  source 1..20: mol_type = other RNA
gtccagaagaagttccagaa

SEQ ID NO: 32 - RNA, 20 nt, synthetic construct
  source 1..20: mol_type = other RNA
tcatgggtgtctgtgggtta

SEQ ID NO: 33 - RNA, 20 nt, synthetic construct
  source 1..20: mol_type = other RNA
gtgggttatttaaaagaaat

SEQ ID NO: 34 - RNA, 20 nt, synthetic construct
  source 1..20: mol_type = other RNA
agttagatgattcacttttt

SEQ ID NO: 35 - RNA, 20 nt, synthetic construct
  source 1..20: mol_type = other RNA
cacttggctggtgtttgact

SEQ ID NO: 36 - RNA, 20 nt, synthetic construct
  source 1..20: mol_type = other RNA
attttgctaaaccattacaa

SEQ ID NO: 37 - RNA, 20 nt, synthetic construct
  source 1..20: mol_type = other RNA
tgcagtgccatcctcatgta

SEQ ID NO: 38 - RNA, 20 nt, synthetic construct
  source 1..20: mol_type = other RNA
catgtcagacttttgtatat

SEQ ID NO: 39 - RNA, 20 nt, synthetic construct
  source 1..20: mol_type = other RNA
ccagaaatacattggtttcg

SEQ ID NO: 40 - RNA, 20 nt, synthetic construct
  source 1..20: mol_type = other RNA
acagaagtgagcaagaagtt

SEQ ID NO: 41 - RNA, 20 nt, synthetic construct
  source 1..20: mol_type = other RNA
ccgggacaccatagactatt

SEQ ID NO: 42 - RNA, 20 nt, synthetic construct
  source 1..20: mol_type = other RNA
gacaccatagactatttgct

SEQ ID NO: 43 - RNA, 20 nt, synthetic construct
  source 1..20: mol_type = other RNA
gaagtgtacaagcaggtgat

SEQ ID NO: 44 - RNA, 20 nt, synthetic construct
  source 1..20: mol_type = other RNA
tgctaaaccattacaatgtt

SEQ ID NO: 45 - RNA, 20 nt, synthetic construct
  source 1..20: mol_type = other RNA
caccatagactatttgcttt

SEQ ID NO: 46 - RNA, 20 nt, synthetic construct
  source 1..20: mol_type = other RNA
attacaatgttaggtctttt

SEQ ID NO: 47 - RNA, 20 nt, synthetic construct
  source 1..20: mol_type = other RNA
cttctgagcagcagattagt

SEQ ID NO: 48 - RNA, 20 nt, synthetic construct
  source 1..20: mol_type = other RNA
gtgtacaagcaggtgatctt

SEQ ID NO: 49 - RNA, 20 nt, synthetic construct
  source 1..20: mol_type = other RNA
cgctactttcgagactactt

SEQ ID NO: 50 - RNA, 20 nt, synthetic construct
  source 1..20: mol_type = other RNA
cattacaatgttaggtcttt

SEQ ID NO: 51 - RNA, 20 nt, synthetic construct
  source 1..20: mol_type = other RNA
gccatcctcatgtacatatt

SEQ ID NO: 52 - RNA, 20 nt, synthetic construct
  source 1..20: mol_type = other RNA
catcctcatgtacatattct

SEQ ID NO: 53 - RNA, 20 nt, synthetic construct
  source 1..20: mol_type = other RNA
gtacatattctgcactgatt

SEQ ID NO: 54 - RNA, 20 nt, synthetic construct
  source 1..20: mol_type = other RNA
tacttcacttggctggtgtt

SEQ ID NO: 55 - RNA, 20 nt, synthetic construct
  source 1..20: mol_type = other RNA
acttcacttggctggtgttt

SEQ ID NO: 56 - RNA, 20 nt, synthetic construct
  source 1..20: mol_type = other RNA
gctactttcgagactacttt

SEQ ID NO: 57 - RNA, 20 nt, synthetic construct
  source 1..20: mol_type = other RNA
cgggacaccatagactattt

SEQ ID NO: 58 - RNA, 20 nt, synthetic construct
  source 1..20: mol_type = other RNA
cggaaccgcaagggctttgt

SEQ ID NO: 59 - RNA, 20 nt, synthetic construct
  source 1..20: mol_type = other RNA
ccattacaatgttaggtctt

SEQ ID NO: 60 - RNA, 20 nt, synthetic construct
  source 1..20: mol_type = other RNA
caatgttaggtcttttttaa

SEQ ID NO: 61 - RNA, 20 nt, synthetic construct
  source 1..20: mol_type = other RNA
gttctaggtggtggctaaat

SEQ ID NO: 62 - RNA, 20 nt, synthetic construct
  source 1..20: mol_type = other RNA
tctaggtggtggctaaatct

SEQ ID NO: 63 - RNA, 20 nt, synthetic construct
  source 1..20: mol_type = other RNA
tggctaaatctgggcctaat

SEQ ID NO: 64 - RNA, 20 nt, synthetic construct
  source 1..20: mol_type = other RNA
ctgaaactgcaggaccagtt

SEQ ID NO: 65 - RNA, 20 nt, synthetic construct
  source 1..20: mol_type = other RNA
gtggagtaactggtttttct

SEQ ID NO: 66 - RNA, 20 nt, synthetic construct
  source 1..20: mol_type = other RNA
cccaagcctcacttttctgt

SEQ ID NO: 67 - RNA, 20 nt, synthetic construct
  source 1..20: mol_type = other RNA
cagtgccatcctcatgtaca

SEQ ID NO: 68 - RNA, 20 nt, synthetic construct
  source 1..20: mol_type = other RNA
agtgccatcctcatgtacat

SEQ ID NO: 69 - RNA, 20 nt, synthetic construct
  source 1..20: mol_type = other RNA
tcatgtacatattctgcact

SEQ ID NO: 70 - RNA, 20 nt, synthetic construct
  source 1..20: mol_type = other RNA
tgcactgattgctggctcat

SEQ ID NO: 71 - RNA, 20 nt, synthetic construct
  source 1..20: mol_type = other RNA
ctctacttcacttggctggt

SEQ ID NO: 72 - RNA, 20 nt, synthetic construct
  source 1..20: mol_type = other RNA
ctgggtgccttctgcaactt

SEQ ID NO: 73 - RNA, 20 nt, synthetic construct
  source 1..20: mol_type = other RNA
tgagggagtacctgatgtct

SEQ ID NO: 74 - RNA, 20 nt, synthetic construct
  source 1..20: mol_type = other RNA
tacctgatgtctggaggtat

SEQ ID NO: 75 - RNA, 20 nt, synthetic construct
  source 1..20: mol_type = other RNA
gccgggacaccatagactat

SEQ ID NO: 76 - RNA, 20 nt, synthetic construct
  source 1..20: mol_type = other RNA
gggacaccatagactatttg

SEQ ID NO: 77 - RNA, 20 nt, synthetic construct
  source 1..20: mol_type = other RNA
acaccatagactatttgctt

SEQ ID NO: 78 - RNA, 20 nt, synthetic construct
  source 1..20: mol_type = other RNA
gctttcaaagaatgggagtg

SEQ ID NO: 79 - RNA, 20 nt, synthetic construct
  source 1..20: mol_type = other RNA
caaagaatgggagtggcaat

SEQ ID NO: 80 - RNA, 20 nt, synthetic construct
  source 1..20: mol_type = other RNA
gaagaagttccagaaataca

SEQ ID NO: 81 - RNA, 20 nt, synthetic construct
  source 1..20: mol_type = other RNA
tggtttcgccccatgcatct

SEQ ID NO: 82 - RNA, 20 nt, synthetic construct
  source 1..20: mol_type = other RNA
ggtttcgccccatgcatctt

SEQ ID NO: 83 - RNA, 20 nt, synthetic construct
  source 1..20: mol_type = other RNA
gctaaaccattacaatgtta

SEQ ID NO: 84 - RNA, 20 nt, synthetic construct
  source 1..20: mol_type = other RNA
tacaatgttaggtctttttt

SEQ ID NO: 85 - RNA, 20 nt, synthetic construct
  source 1..20: mol_type = other RNA
acaatgttaggtctttttta

SEQ ID NO: 86 - RNA, 20 nt, synthetic construct
  source 1..20: mol_type = other RNA
tgttaggtcttttttaagaa

SEQ ID NO: 87 - RNA, 20 nt, synthetic construct
  source 1..20: mol_type = other RNA
cacttctcatacaagcccct

SEQ ID NO: 88 - RNA, 20 nt, synthetic construct
  source 1..20: mol_type = other RNA
actgcaggaccagtttctct

SEQ ID NO: 89 - RNA, 20 nt, synthetic construct
  source 1..20: mol_type = other RNA
ctctgccaaggggaggagtt

SEQ ID NO: 90 - RNA, 20 nt, synthetic construct
  source 1..20: mol_type = other RNA
accatgagctaggtggagta

SEQ ID NO: 91 - RNA, 20 nt, synthetic construct
  source 1..20: mol_type = other RNA
ccatgagctaggtggagtaa

SEQ ID NO: 92 - RNA, 20 nt, synthetic construct
  source 1..20: mol_type = other RNA
gctaggtggagtaactggtt

SEQ ID NO: 93 - RNA, 20 nt, synthetic construct
  source 1..20: mol_type = other RNA
ggtggagtaactggtttttc

SEQ ID NO: 94 - RNA, 20 nt, synthetic construct
  source 1..20: mol_type = other RNA
gcagcagattagttccaaag

SEQ ID NO: 95 - RNA, 20 nt, synthetic construct
  source 1..20: mol_type = other RNA
gattagttccaaagcaggtg

SEQ ID NO: 96 - RNA, 20 nt, synthetic construct
  source 1..20: mol_type = other RNA
ccgaacccaagcctcacttt

SEQ ID NO: 97 - RNA, 22 nt, synthetic construct
  source 1..22: mol_type = other RNA
aacttcttctggacccatcggc

SEQ ID NO: 98 - RNA, 22 nt, synthetic construct
  source 1..22: mol_type = other RNA
ataatttcttttaaataaccca

SEQ ID NO: 99 - RNA, 22 nt, synthetic construct
  source 1..22: mol_type = other RNA
atagttcctggtggtcagcagg

SEQ ID NO: 100 - RNA, 22 nt, synthetic construct
  source 1..22: mol_type = other RNA
agatatagttcctggtggtcag

SEQ ID NO: 101 - RNA, 22 nt, synthetic construct
  source 1..22: mol_type = other RNA
aataacccacagacacccatga

SEQ ID NO: 102 - RNA, 22 nt, synthetic construct
  source 1..22: mol_type = other RNA
aaataacccacagacacccatg

SEQ ID NO: 103 - RNA, 22 nt, synthetic construct
  source 1..22: mol_type = other RNA
taaataacccacagacacccat

SEQ ID NO: 104 - RNA, 22 nt, synthetic construct
  source 1..22: mol_type = other RNA
tttaaataacccacagacaccc

SEQ ID NO: 105 - RNA, 22 nt, synthetic construct
  source 1..22: mol_type = other RNA
aatttcttttaaataacccaca

SEQ ID NO: 106 - RNA, 22 nt, synthetic construct
  source 1..22: mol_type = other RNA
taatttcttttaaataacccac

SEQ ID NO: 107 - RNA, 22 nt, synthetic construct
  source 1..22: mol_type = other RNA
atatagttcctggtggtcagca

SEQ ID NO: 108 - RNA, 22 nt, synthetic construct
  source 1..22: mol_type = other RNA
aagatatagttcctggtggtca

SEQ ID NO: 109 - RNA, 22 nt, synthetic construct
  source 1..22: mol_type = other RNA
aaagatatagttcctggtggtc

SEQ ID NO: 110 - RNA, 22 nt, synthetic construct
  source 1..22: mol_type = other RNA
atccaaagatatagttcctggt

SEQ ID NO: 111 - RNA, 22 nt, synthetic construct
  source 1..22: mol_type = other RNA
atgatagcattgccactcccat

SEQ ID NO: 112 - RNA, 22 nt, synthetic construct
  source 1..22: mol_type = other RNA
ataacccacagacacccatgac

SEQ ID NO: 113 - RNA, 22 nt, synthetic construct
  source 1..22: mol_type = other RNA
ttaaataacccacagacaccca

SEQ ID NO: 114 - RNA, 22 nt, synthetic construct
  source 1..22: mol_type = other RNA
ttttaaataacccacagacacc

SEQ ID NO: 115 - RNA, 22 nt, synthetic construct
  source 1..22: mol_type = other RNA
cttttaaataacccacagacac

SEQ ID NO: 116 - RNA, 22 nt, synthetic construct
  source 1..22: mol_type = other RNA
ttcttttaaataacccacagac

SEQ ID NO: 117 - RNA, 22 nt, synthetic construct
  source 1..22: mol_type = other RNA
agctggatgggaaagtagtctc

SEQ ID NO: 118 - RNA, 22 nt, synthetic construct
  source 1..22: mol_type = other RNA
aggttgtgtgtcttcaccagct

SEQ ID NO: 119 - RNA, 22 nt, synthetic construct
  source 1..22: mol_type = other RNA
agcaggttgtgtgtcttcacca

SEQ ID NO: 120 - RNA, 22 nt, synthetic construct
  source 1..22: mol_type = other RNA
agttcctggtggtcagcaggtt

SEQ ID NO: 121 - RNA, 22 nt, synthetic construct
  source 1..22: mol_type = other RNA
tatagttcctggtggtcagcag

SEQ ID NO: 122 - RNA, 22 nt, synthetic construct
  source 1..22: mol_type = other RNA
tagcattgccactcccattctt

SEQ ID NO: 123 - RNA, 22 nt, synthetic construct
  source 1..22: mol_type = other RNA
tgatgatagcattgccactccc

SEQ ID NO: 124 - RNA, 22 nt, synthetic construct
  source 1..22: mol_type = other RNA
atgatgatagcattgccactcc

SEQ ID NO: 125 - RNA, 22 nt, synthetic construct
  source 1..22: mol_type = other RNA
acgatgatgatagcattgccac

SEQ ID NO: 126 - RNA, 22 nt, synthetic construct
  source 1..22: mol_type = other RNA
ttcttgccaggcatggagctca

SEQ ID NO: 127 - RNA, 22 nt, synthetic construct
  source 1..22: mol_type = other RNA
ttctggaacttcttctggaccc

SEQ ID NO: 128 - RNA, 22 nt, synthetic construct
  source 1..22: mol_type = other RNA
taacccacagacacccatgaca

SEQ ID NO: 129 - RNA, 22 nt, synthetic construct
  source 1..22: mol_type = other RNA
atttcttttaaataacccacag

SEQ ID NO: 130 - RNA, 22 nt, synthetic construct
  source 1..22: mol_type = other RNA
aaaaagtgaatcatctaactgg

SEQ ID NO: 131 - RNA, 22 nt, synthetic construct
  source 1..22: mol_type = other RNA
agtcaaacaccagccaagtgaa

SEQ ID NO: 132 - RNA, 22 nt, synthetic construct
  source 1..22: mol_type = other RNA
ttgtaatggtttagcaaaattg

SEQ ID NO: 133 - RNA, 22 nt, synthetic construct
  source 1..22: mol_type = other RNA
tacatgaggatggcactgcagg

SEQ ID NO: 134 - RNA, 22 nt, synthetic construct
  source 1..22: mol_type = other RNA
atatacaaaagtctgacatggt

SEQ ID NO: 135 - RNA, 22 nt, synthetic construct
  source 1..22: mol_type = other RNA
cgaaaccaatgtatttctggaa

SEQ ID NO: 136 - RNA, 22 nt, synthetic construct
  source 1..22: mol_type = other RNA
aacttcttgctcacttctgtgg

SEQ ID NO: 137 - RNA, 22 nt, synthetic construct
  source 1..22: mol_type = other RNA
aatagtctatggtgtcccggct

SEQ ID NO: 138 - RNA, 22 nt, synthetic construct
  source 1..22: mol_type = other RNA
agcaaatagtctatggtgtccc

SEQ ID NO: 139 - RNA, 22 nt, synthetic construct
  source 1..22: mol_type = other RNA
atcacctgcttgtacacttcat

SEQ ID NO: 140 - RNA, 22 nt, synthetic construct
  source 1..22: mol_type = other RNA
aacattgtaatggtttagcaaa

SEQ ID NO: 141 - RNA, 22 nt, synthetic construct
  source 1..22: mol_type = other RNA
aaagcaaatagtctatggtgtc

SEQ ID NO: 142 - RNA, 22 nt, synthetic construct
  source 1..22: mol_type = other RNA
aaaagacctaacattgtaatgg

SEQ ID NO: 143 - RNA, 22 nt, synthetic construct
  source 1..22: mol_type = other RNA
actaatctgctgctcagaaggc

SEQ ID NO: 144 - RNA, 22 nt, synthetic construct
  source 1..22: mol_type = other RNA
aagatcacctgcttgtacactt

SEQ ID NO: 145 - RNA, 22 nt, synthetic construct
  source 1..22: mol_type = other RNA
aagtagtctcgaaagtagcgcc

SEQ ID NO: 146 - RNA, 22 nt, synthetic construct
  source 1..22: mol_type = other RNA
aaagacctaacattgtaatggt

SEQ ID NO: 147 - RNA, 22 nt, synthetic construct
  source 1..22: mol_type = other RNA
aatatgtacatgaggatggcac

SEQ ID NO: 148 - RNA, 22 nt, synthetic construct
  source 1..22: mol_type = other RNA
agaatatgtacatgaggatggc

SEQ ID NO: 149 - RNA, 22 nt, synthetic construct
  source 1..22: mol_type = other RNA
aatcagtgcagaatatgtacat

SEQ ID NO: 150 - RNA, 22 nt, synthetic construct
  source 1..22: mol_type = other RNA
aacaccagccaagtgaagtaga

SEQ ID NO: 151 - RNA, 22 nt, synthetic construct
  source 1..22: mol_type = other RNA
aaacaccagccaagtgaagtag

SEQ ID NO: 152 - RNA, 22 nt, synthetic construct
  source 1..22: mol_type = other RNA
aaagtagtctcgaaagtagcgc

SEQ ID NO: 153 - RNA, 22 nt, synthetic construct
  source 1..22: mol_type = other RNA
aaatagtctatggtgtcccggc

SEQ ID NO: 154 - RNA, 22 nt, synthetic construct
  source 1..22: mol_type = other RNA
acaaagcccttgcggttccgca

SEQ ID NO: 155 - RNA, 22 nt, synthetic construct
  source 1..22: mol_type = other RNA
aagacctaacattgtaatggtt

SEQ ID NO: 156 - RNA, 22 nt, synthetic construct
  source 1..22: mol_type = other RNA
ttaaaaaagacctaacattgta

SEQ ID NO: 157 - RNA, 22 nt, synthetic construct
  source 1..22: mol_type = other RNA
atttagccaccacctagaacag

SEQ ID NO: 158 - RNA, 22 nt, synthetic construct
  source 1..22: mol_type = other RNA
agatttagccaccacctagaac

SEQ ID NO: 159 - RNA, 22 nt, synthetic construct
  source 1..22: mol_type = other RNA
attaggcccagatttagccacc

SEQ ID NO: 160 - RNA, 22 nt, synthetic construct
  source 1..22: mol_type = other RNA
aactggtcctgcagtttcagga

SEQ ID NO: 161 - RNA, 22 nt, synthetic construct
  source 1..22: mol_type = other RNA
agaaaaaccagttactccacct

SEQ ID NO: 162 - RNA, 22 nt, synthetic construct
  source 1..22: mol_type = other RNA
acagaaaagtgaggcttgggtt

SEQ ID NO: 163 - RNA, 22 nt, synthetic construct
  source 1..22: mol_type = other RNA
tgtacatgaggatggcactgca

SEQ ID NO: 164 - RNA, 22 nt, synthetic construct
  source 1..22: mol_type = other RNA
atgtacatgaggatggcactgc

SEQ ID NO: 165 - RNA, 22 nt, synthetic construct
  source 1..22: mol_type = other RNA
agtgcagaatatgtacatgagg

SEQ ID NO: 166 - RNA, 22 nt, synthetic construct
  source 1..22: mol_type = other RNA
atgagccagcaatcagtgcaga

SEQ ID NO: 167 - RNA, 22 nt, synthetic construct
  source 1..22: mol_type = other RNA
accagccaagtgaagtagagca

SEQ ID NO: 168 - RNA, 22 nt, synthetic construct
  source 1..22: mol_type = other RNA
aagttgcagaaggcacccaggc

SEQ ID NO: 169 - RNA, 22 nt, synthetic construct
  source 1..22: mol_type = other RNA
agacatcaggtactccctcaac

SEQ ID NO: 170 - RNA, 22 nt, synthetic construct
  source 1..22: mol_type = other RNA
atacctccagacatcaggtact

SEQ ID NO: 171 - RNA, 22 nt, synthetic construct
  source 1..22: mol_type = other RNA
atagtctatggtgtcccggctg

SEQ ID NO: 172 - RNA, 22 nt, synthetic construct
  source 1..22: mol_type = other RNA
caaatagtctatggtgtcccgg

SEQ ID NO: 173 - RNA, 22 nt, synthetic construct
  source 1..22: mol_type = other RNA
aagcaaatagtctatggtgtcc

SEQ ID NO: 174 - RNA, 22 nt, synthetic construct
  source 1..22: mol_type = other RNA
cactcccattctttgaaagcaa

SEQ ID NO: 175 - RNA, 22 nt, synthetic construct
  source 1..22: mol_type = other RNA
attgccactcccattctttgaa

SEQ ID NO: 176 - RNA, 22 nt, synthetic construct
  source 1..22: mol_type = other RNA
tgtatttctggaacttcttctg

SEQ ID NO: 177 - RNA, 22 nt, synthetic construct
  source 1..22: mol_type = other RNA
agatgcatggggcgaaaccaat

SEQ ID NO: 178 - RNA, 22 nt, synthetic construct
  source 1..22: mol_type = other RNA
aagatgcatggggcgaaaccaa

SEQ ID NO: 179 - RNA, 22 nt, synthetic construct
  source 1..22: mol_type = other RNA
taacattgtaatggtttagcaa

SEQ ID NO: 180 - RNA, 22 nt, synthetic construct
  source 1..22: mol_type = other RNA
aaaaaagacctaacattgtaat

SEQ ID NO: 181 - RNA, 22 nt, synthetic construct
  source 1..22: mol_type = other RNA
taaaaaagacctaacattgtaa

SEQ ID NO: 182 - RNA, 22 nt, synthetic construct
  source 1..22: mol_type = other RNA
ttcttaaaaaagacctaacatt

SEQ ID NO: 183 - RNA, 22 nt, synthetic construct
  source 1..22: mol_type = other RNA
aggggcttgtatgagaagtggc

SEQ ID NO: 184 - RNA, 22 nt, synthetic construct
  source 1..22: mol_type = other RNA
agagaaactggtcctgcagttt

SEQ ID NO: 185 - RNA, 22 nt, synthetic construct
  source 1..22: mol_type = other RNA
aactcctccccttggcagagaa

SEQ ID NO: 186 - RNA, 22 nt, synthetic construct
  source 1..22: mol_type = other RNA
tactccacctagctcatggtgg

SEQ ID NO: 187 - RNA, 22 nt, synthetic construct
  source 1..22: mol_type = other RNA
ttactccacctagctcatggtg

SEQ ID NO: 188 - RNA, 22 nt, synthetic construct
  source 1..22: mol_type = other RNA
aaccagttactccacctagctc

SEQ ID NO: 189 - RNA, 22 nt, synthetic construct
  source 1..22: mol_type = other RNA
gaaaaaccagttactccaccta

SEQ ID NO: 190 - RNA, 22 nt, synthetic construct
  source 1..22: mol_type = other RNA
ctttggaactaatctgctgctc

SEQ ID NO: 191 - RNA, 22 nt, synthetic construct
  source 1..22: mol_type = other RNA
cacctgctttggaactaatctg

SEQ ID NO: 192 - RNA, 22 nt, synthetic construct
  source 1..22: mol_type = other RNA
aaagtgaggcttgggttcgggg

SEQ ID NO: 193 - RNA, 2407 nt, Homo sapiens
  source 1..2407: mol_type = mRNA
gccgcggctgccgcctctgctggggtctaggctgtttctctcgcgccaccactggccgccggccgcagctccaggtgtcctagccgcccagcctcgacgccgtcccgggacccctgtgctctgcgcgaagccctggccccgggggccggggcatgggccaggggcgcggggtgaagcggcttcccgcggggccgtgactgggcgggcttcagccatgaagaccctcatagccgcctactccggggtcctgcgcggcgagcgtcaggccgaggctgaccggagccagcgctctcacggaggacctgcgctgtcgcgcgaggggtctgggagatggggcactggatccagcatcctctccgccctccaggacctcttctctgtcacctggctcaataggtccaaggtggaaaagcagctacaggtcatctcagtgctccagtgggtcctgtccttccttgtactgggagtggcctgcagtgccatcctcatgtacatattctgcactgattgctggctcatcgctgtgctctacttcacttggctggtgtttgactggaacacacccaagaaaggtggcaggaggtcacagtgggtccgaaactgggctgtgtggcgctactttcgagactactttcccatccagctggtgaagacacacaacctgctgaccaccaggaactatatctttggataccacccccatggtatcatgggcctgggtgccttctgcaacttcagcacagaggccacagaagtgagcaagaagttcccaggcatacggccttacctggctacactggcaggcaacttccgaatgcctgtgttgagggagtacctgatgtctggaggtatctgccctgtcagccgggacaccatagactatttgctttcaaagaatgggagtggcaatgctatcatcatcgtggtcgggggtgcggctgagtctctgagctccatgcctggcaagaatgcagtcaccctgcggaaccgcaagggctttgtgaaactggccctgcgtcatggagctgacctggttcccatctactcctttggagagaatgaagtgtacaagcaggtgatcttcgaggagggctcctggggccgatgggtccagaagaagttccagaaatacattggtttcgccccatgcatcttccatggtcgaggcctcttctcctccgacacctgggggctggtgccctactccaagcccatcaccactgttgtgggagagcccatcaccatccccaagctggagcacccaacccagcaagacatcgacctgtaccacaccatgtacatggaggccctggtgaagctcttcgacaagcacaagaccaagttcggcctcccggagactgaggtcctggaggtgaactgagccagccttcggggccaattccctggaggaaccagctgcaaatcacttttttgctctgtaaatttggaagtgtcatgggtgtctgtgggttatttaaaagaaattataacaattttgctaaaccattacaatgttaggtcttttttaagaaggaaaaagtcagtatttcaagttctttcacttccagcttgccctgttctaggtggtggctaaatctgggcctaatctgggtggctcagctaacctctcttcttcccttcctgaagtgacaaaggaaactcagtcttcttggggaagaaggattgccattagtgacttggaccagttagatgattcactttttgcccctagggatgagaggcgaaagccacttctcatacaagcccctttattgccactaccccacgctcgtctagtcctgaaactgcaggaccagtttctctgccaaggggaggagttggagagcacagttgccccgttgtgtgagggcagtagtaggcatctggaatgctccagtttgatctcccttctgccacccctacctcacccctagtcactcatatcggagcctggactggcctccaggatgaggatgggggtggcaatgacaccctgcaggggaaaggactgccccccatgcaccattgcagggaggatgccgccaccatgagctaggtggagtaactggtttttcttgggtggctgatgacatggatgcagcacagactcagccttggcctggagcacatgcttactggtggcctcagtttaccttccccagatcctagattctggatgtgaggaagagatccctcttcagaaggggcctggccttctgagcagcagattagttccaaagcaggtggcccccgaacccaagcctcacttttctgtgccttcctgagggggttgggccggggaggaaacccaaccctctcctgtgtgttctgttatctcttgatgagatcattgcaccatgtcagacttttgtatatgccttgaaaataaatgaaagtgagaatcctc

SEQ ID NO: 194 - RNA, 20 nt, synthetic construct
  source 1..20: mol_type = other RNA
aagcaaatagtctatggtgt

SEQ ID NO: 195 - RNA, 21 nt, synthetic construct
  source 1..21: mol_type = other RNA
taagcaaatagtctatggtgt

SEQ ID NO: 196 - RNA, 20 nt, synthetic construct
  source 1..20: mol_type = other RNA
ttaaataacccacagacacc

SEQ ID NO: 197 - RNA, 21 nt, synthetic construct
  source 1..21: mol_type = other RNA
tttaaataacccacagacacc

SEQ ID NO: 198 - RNA, 20 nt, synthetic construct
  source 1..20: mol_type = other RNA
tgtatttctggaacttcttc

SEQ ID NO: 199 - RNA, 21 nt, synthetic construct
  source 1..21: mol_type = other RNA
ttgtatttctggaacttcttc

SEQ ID NO: 200 - RNA, 21 nt, synthetic construct
  source 1..21: mol_type = other RNA
aaagcaaatagtctatggtgt

SEQ ID NO: 201 - RNA, 21 nt, synthetic construct
  source 1..21: mol_type = other RNA
acaccatagactatttgcttt